European Patent Specification EP 3 845 643 B1, published March 20, 2024. Title: NOVEL FRUCTOSE-C4-EPIMERASE AND METHOD OF PREPARING TAGATOSE USING THE SAME. Applicant: CJ CheilJedang Corporation. The sequence listing filed with the application follows.

SEQUENCE LISTING (2 sequences)

SEQ ID NO: 1 - protein, 431 aa, Unknown
  Litorilinea aerophila
MYPVLENILRAQQQGEALGIPSICSAHPFVLEATFRHALTTGRTVLIESTCNQVNQHGGYTGMTPGDFVAYVAALADRLHFPRERILLGGDHLGPNPWRDRPADQALNQARILVQEYVRAGYGKIHLDASMACGGDPADAPLDKAVAAERAAALAEAAEAAFQRMGSGTPPCYVIGTEVPPPGGAQGDDMPLAITAPREVAETIELTQAAFRRRGLEAAWERVIAVVVQPGVEFGDEQVHPYDRAAAAGLARAIEPYGRLVYEAHSTDYQTRQALRDLVADHFAILKVGPALTFAFREAVFALAAVEEEWLAGQAGVVLSRLREELEAAMIQDPTHWRGYYRGDERHQRLARRYSYSDRARYYWPRPSVQAALERLLHNLEAAPPPLTLLSQYLPVQYWSVREGLLEPTPRSLIVDKIIQVLNDYTWACGG

SEQ ID NO: 2 - DNA, 1296 bp, Unknown
  Litorilinea aerophila
atgtaccccgtcctggaaaacatcctgcgcgcccagcagcagggcgaagccctgggcatcccgtccatctgctccgcgcacccttttgtgctggaggcgactttccgccacgccctgaccaccggccggaccgtgctcattgaatccacctgcaaccaggtgaaccagcacggcggatacacgggcatgacgcccggtgactttgtggcctacgtggccgccctggccgatcggctccactttccccgagaacgcatcctgttgggtggcgatcacctggggcccaacccctggcgggatcgcccggcggaccaggccctgaaccaggcccggatcctggtccaggaatatgtacgggccggctacggcaagatccacctggacgcgagcatggcctgtggcggggatccagccgacgcccccctggacaaagccgtggcggccgagcgggccgcagccctggccgaggcagcggaagccgcgtttcaacggatggggagtggaacgcccccctgctacgtcatcggcacggaggtgccacccccgggcggcgcccagggagacgacatgcccctggccatcaccgcgccccgggaagtggccgagaccatcgagctgacccaggcagccttccgccggcgcgggctggaagcagcctgggaacgggtcattgcggtggtggtgcagccaggcgtggagttcggcgacgagcaggtgcatccatatgaccgggctgcggcggccggcctggcccgggccatcgagccctacgggcggctggtgtacgaggcccactccaccgactaccagacccgccaggccctgcgggatctggtggcggatcactttgccatcctgaaggtggggccggccctcacttttgcctttcgggaggcggtctttgccctggctgcggtggaggaggaatggctggccggccaggcgggggtggtcctgtcccggctgcgggaggagctggaggcagccatgatccaggatcccacccactggcggggctattatcgaggggatgagcggcatcaacgattggctcgccgctacagctacagcgaccgggcccgctactattggccacggccgtccgtccaggcggcgctggaacggctgctacacaacctggaggccgccccgccgcccctgaccctgctcagccaatacctgcctgtgcagtactggagcgtccgcgaagggctcctggagccgacgccccggtccctgatcgtggacaaaatcatccaggtgttgaatgactacacctgggcctgtgggggatga